European Patent Specification EP 3 757 123 B1, published August 21, 2024. Title: MUTATED IMMUNOGLOBULIN-BINDING POLYPEPTIDES. Applicant: GE Healthcare Bio-Sciences AB. The sequence listing filed with the application follows.

SEQUENCE LISTING (53 sequences)

SEQ ID NO: 1 - protein, 51 aa, Staphylococcus aureus
AQQNAFYQVLNMPNLNADQRNGFIQSLKDDPSQSANVLGEAQKLNDSQAPK

SEQ ID NO: 2 - protein, 61 aa, Staphylococcus aureus
ADAQQNKFNKDQQSAFYEILNMPNLNEEQRNGFIQSLKDDPSQSTNVLGEAKKLNESQAPK

SEQ ID NO: 3 - protein, 58 aa, Staphylococcus aureus
ADNNFNKEQQNAFYEILNMPNLNEEQRNGFIQSLKDDPSQSANLLAEAKKLNESQAPK

SEQ ID NO: 4 - protein, 58 aa, Staphylococcus aureus [sequence omitted]

SEQ ID NO: 5 - protein, 58 aa, Staphylococcus aureus
ADNKFNKEQQNAFYEILHLPNLTEEQRNGFIQSLKDDPSVSKEILAEAKKLNDAQAPK

SEQ ID NO: 6 - protein, 58 aa, Escherichia coli [sequence omitted]

SEQ ID NO: 7 - protein, 58 aa, Escherichia coli [sequence omitted]

SEQ ID NO: 8 - protein, 58 aa, Escherichia coli
VDAKFDKEAQEAFYEILHLPNLTEEQRNAFIQSLKDDPSQSAALLAEAKKLNDAQAPK

SEQ ID NO: 9 - protein, 58 aa, Escherichia coli
VDAKFDKEAQEAFYEILHLPNLTEEQRAAFIQSLKDDPSQSAALLAEAKKLNDAQAPK

SEQ ID NO: 10 - protein, 58 aa, Escherichia coli
VDAKFDKEAQEAFYEILHLPNLTEEQRNAFIQSLKDDPSVSKEILAEAKKLNDAQAPK

SEQ ID NO: 11 - protein, 58 aa, Escherichia coli
VDAKFDKEAQEAFYEILHLPNLTEEQRNAFIQSLKDDPSVSKAILAEAKKLNDAQAPK

SEQ ID NO: 12 - protein, 58 aa, Escherichia coli
VDAKFDKEQQEAFYEILHLPNLTEEQRNAFIASLKDDPSQSANLLAEAKKLNDAQAPK

SEQ ID NO: 13 - protein, 58 aa, Escherichia coli
VDAKFDKEQQEAFYEILHLPNLTEEQRNAFIQSLKDDPSQSANLLAEAKKLNDAQAPK

SEQ ID NO: 14 - protein, 58 aa, Escherichia coli
VDAKFDKEQQEAFYEILHLPNLTEEQRNAFIESLKDDPSESANLLAEAKKLNDAQAPK

SEQ ID NO: 15 - protein, 58 aa, Escherichia coli
VDAKFDKEQQEAFYEILHLPNLTEEQRNAFIESLKDDPSQSANLLAEAKRLNDAQAPK

SEQ ID NO: 16 - protein, 58 aa, Escherichia coli
VDAKFDKEQQKAFYEILHLPNLTEEQRNAFIQSLKDDPSQSANLLAEAKKLNDAQAPK

SEQ ID NO: 17 - protein, 237 aa, Escherichia coli
AQGTVDAKFDKEAQEAFYEILHLPNLTEEQRNAFIQSLKDDPSQSAALLAEAKKLNDAQAPKVDAKFDKEAQEAFYEILHLPNLTEEQRNAFIQSLKDDPSQSAALLAEAKKLNDAQAPKVDAKFDKEAQEAFYEILHLPNLTEEQRNAFIQSLKDDPSQSAALLAEAKKLNDAQAPKVDAKFDKEAQEAFYEILHLPNLTEEQRNAFIQSLKDDPSQSAALLAEAKKLNDAQAPKC

SEQ ID NO: 18 - protein, 237 aa, Escherichia coli
AQGTVDAKFDKEAQEAFYEILHLPNLTEEQRAAFIQSLKDDPSQSAALLAEAKKLNDAQAPKVDAKFDKEAQEAFYEILHLPNLTEEQRAAFIQSLKDDPSQSAALLAEAKKLNDAQAPKVDAKFDKEAQEAFYEILHLPNLTEEQRAAFIQSLKDDPSQSAALLAEAKKLNDAQAPKVDAKFDKEAQEAFYEILHLPNLTEEQRAAFIQSLKDDPSQSAALLAEAKKLNDAQAPKC

SEQ ID NO: 19 - protein, 237 aa, Escherichia coli
AQGTVDAKFDKEAQEAFYEILHLPNLTEEQRNAFIQSLKDDPSVSKEILAEAKKLNDAQAPKVDAKFDKEAQEAFYEILHLPNLTEEQRNAFIQSLKDDPSVSKEILAEAKKLNDAQAPKVDAKFDKEAQEAFYEILHLPNLTEEQRNAFIQSLKDDPSVSKEILAEAKKLNDAQAPKVDAKFDKEAQEAFYEILHLPNLTEEQRNAFIQSLKDDPSVSKEILAEAKKLNDAQAPKC

SEQ ID NO: 20 - protein, 237 aa, Escherichia coli
AQGTVDAKFDKEAQEAFYEILHLPNLTEEQRNAFIQSLKDDPSVSKAILAEAKKLNDAQAPKVDAKFDKEAQEAFYEILHLPNLTEEQRNAFIQSLKDDPSVSKAILAEAKKLNDAQAPKVDAKFDKEAQEAFYEILHLPNLTEEQRNAFIQSLKDDPSVSKAILAEAKKLNDAQAPKVDAKFDKEAQEAFYEILHLPNLTEEQRNAFIQSLKDDPSVSKAILAEAKKLNDAQAPKC

SEQ ID NO: 21 - protein, 237 aa, Escherichia coli
AQGTVDAKFDKEQQNAFYEILHLPNLTEEQRNAFIQSLKDDPSQSANLLAEAKKLNDAQAPKVDAKFDKEQQNAFYEILHLPNLTEEQRNAFIQSLKDDPSQSANLLAEAKKLNDAQAPKVDAKFDKEQQNAFYEILHLPNLTEEQRNAFIQSLKDDPSQSANLLAEAKKLNDAQAPKVDAKFDKEQQNAFYEILHLPNLTEEQRNAFIQSLKDDPSQSANLLAEAKKLNDAQAPKC

SEQ ID NO: 22 - protein, 58 aa, Staphylococcus aureus
ADNNFNKEQQNAFYEILNMPNLNEEQRNGFIQSLKDDPSQSANLLSEAKKLNESQAPK

SEQ ID NO: 23 - protein, 58 aa, Escherichia coli
VDAKFDKEQQKAFYEILKLPNLTEEQRNAFIQKLKDEPSQSRAILAEAKRYNDAQAPK

SEQ ID NO: 24 - protein, 58 aa, Escherichia coli
VDAKFDKEAQEAFYEILHLPNLTEEQRAAFIQSLKDDPSVSKAILAEAKKLNDAQAPK

SEQ ID NO: 25 - protein, 58 aa, Escherichia coli
VDAKFDKEAQKAFYEILKLPNLTEEQRAAFIQKLKDEPSQSRAILAEAKRYNDAQAPK

SEQ ID NO: 26 - protein, 58 aa, Escherichia coli
VDAKFDKEQQKAFYEILKLPNLTEEQRNAFIQSLKDEPSQSRAILAEAKKLNDAQAPK

SEQ ID NO: 27 - protein, 58 aa, Escherichia coli
VDAKFDKEAQKAFYEILKLPNLTEEQRNAFIQSLKDEPSQSRAILAEAKKLNDAQAPK

SEQ ID NO: 28 - protein, 58 aa, Escherichia coli
VDAKFDKEAQKAFYEILKLPNLTEEQRNAFIQSLKDEPSQSRAILAEAKRLNDAQAPK

SEQ ID NO: 29 - protein, 58 aa, Escherichia coli
VDAKFDKEAQKAFYEILKLPNLTEEQRNAFIQSLKDEPSQSRNLLAEAKKLNDAQAPK

SEQ ID NO: 30 - protein, 237 aa, Escherichia coli
AQGTVDAKFDKEQQKAFYEILKLPNLTEEQRNAFIQKLKDEPSQSRAILAEAKRYNDAQAPKVDAKFDKEQQKAFYEILKLPNLTEEQRNAFIQKLKDEPSQSRAILAEAKRYNDAQAPKVDAKFDKEQQKAFYEILKLPNLTEEQRNAFIQKLKDEPSQSRAILAEAKRYNDAQAPKVDAKFDKEQQKAFYEILKLPNLTEEQRNAFIQKLKDEPSQSRAILAEAKRYNDAQAPKC

SEQ ID NO: 31 - protein, 237 aa, Escherichia coli
AQGTVDAKFDKEAQKAFYEILKLPNLTEEQRNAFIQSLKDEPSQSRNLLAEAKKLNDAQAPKVDAKFDKEAQKAFYEILKLPNLTEEQRNAFIQSLKDEPSQSRNLLAEAKKLNDAQAPKVDAKFDKEAQKAFYEILKLPNLTEEQRNAFIQSLKDEPSQSRNLLAEAKKLNDAQAPKVDAKFDKEAQKAFYEILKLPNLTEEQRNAFIQSLKDEPSQSRNLLAEAKKLNDAQAPKC

SEQ ID NO: 32 - protein, 237 aa, Escherichia coli
AQGTVDAKFDKEAQEAFYEILHLPNLTEEQRAAFIQSLKDDPSVSKAILAEAKKLNDAQAPKVDAKFDKEAQEAFYEILHLPNLTEEQRAAFIQSLKDDPSVSKAILAEAKKLNDAQAPKVDAKFDKEAQEAFYEILHLPNLTEEQRAAFIQSLKDDPSVSKAILAEAKKLNDAQAPKVDAKFDKEAQEAFYEILHLPNLTEEQRAAFIQSLKDDPSVSKAILAEAKKLNDAQAPKC

SEQ ID NO: 33 - protein, 353 aa, Escherichia coli
AQGTVDAKFDKEAQEAFYEILHLPNLTEEQRNAFIQSLKDDPSVSKAILAEAKKLNDAQAPKVDAKFDKEAQEAFYEILHLPNLTEEQRNAFIQSLKDDPSVSKAILAEAKKLNDAQAPKVDAKFDKEAQEAFYEILHLPNLTEEQRNAFIQSLKDDPSVSKAILAEAKKLNDAQAPKVDAKFDKEAQEAFYEILHLPNLTEEQRNAFIQSLKDDPSVSKAILAEAKKLNDAQAPKVDAKFDKEAQEAFYEILHLPNLTEEQRNAFIQSLKDDPSVSKAILAEAKKLNDAQAPKVDAKFDKEAQEAFYEILHLPNLTEEQRNAFIQSLKDDPSVSKAILAEAKKLNDAQAPKC

SEQ ID NO: 34 - protein, 237 aa, Escherichia coli
AQGTVDAKFDKEAQEAFYEILHLPNLTEEQRNAFIQSLKDEPSVSKAILAEAKKLNDAQAPKVDAKFDKEAQEAFYEILHLPNLTEEQRNAFIQSLKDEPSVSKAILAEAKKLNDAQAPKVDAKFDKEAQEAFYEILHLPNLTEEQRNAFIQSLKDEPSVSKAILAEAKKLNDAQAPKVDAKFDKEAQEAFYEILHLPNLTEEQRNAFIQSLKDEPSVSKAILAEAKKLNDAQAPKC

SEQ ID NO: 35 - protein, 237 aa, Escherichia coli
AQGTVDAKFDKEAQEAFYEILHLPNLTEEQRNAFIQSLKDEPSVSRAILAEAKKLNDAQAPKVDAKFDKEAQEAFYEILHLPNLTEEQRNAFIQSLKDEPSVSRAILAEAKKLNDAQAPKVDAKFDKEAQEAFYEILHLPNLTEEQRNAFIQSLKDEPSVSRAILAEAKKLNDAQAPKVDAKFDKEAQEAFYEILHLPNLTEEQRNAFIQSLKDEPSVSRAILAEAKKLNDAQAPKC

SEQ ID NO: 36 - protein, 58 aa, Escherichia coli
ADNKFNKEAQEAFYEILHLPNLNEEQRNGFIQSLKDDPSVSKAILAEAKKLNDAQAPK

SEQ ID NO: 37 - protein, 58 aa, Escherichia coli
ADNKFNKEAQEAFYEILHLPNLTEEQRNGFIQSLKDDPSVSKAILAEAKKLNDAQAPK

SEQ ID NO: 38 - protein, 58 aa, Escherichia coli
VDAKFDKEQQYAFYEILHLPNLTEEQRNAFIQSLKDDPSQSANLLAEAKKLNDAQAPK

SEQ ID NO: 39 - protein, 58 aa, Escherichia coli
VDAKFDKEQQTAFYEILHLPNLTEEQRNAFIQSLKDDPSQSANLLAEAKKLNDAQAPK

SEQ ID NO: 40 - protein, 58 aa, Escherichia coli
VDAKFDKEQQFAFYEILHLPNLTEEQRNAFIQSLKDDPSQSANLLAEAKKLNDAQAPK

SEQ ID NO: 41 - protein, 58 aa, Escherichia coli
VDAKFDKEQQLAFYEILHLPNLTEEQRNAFIQSLKDDPSQSANLLAEAKKLNDAQAPK

SEQ ID NO: 42 - protein, 58 aa, Escherichia coli
VDAKFDKEQQWAFYEILHLPNLTEEQRNAFIQSLKDDPSQSANLLAEAKKLNDAQAPK

SEQ ID NO: 43 - protein, 58 aa, Escherichia coli
VDAKFDKEQQIAFYEILHLPNLTEEQRNAFIQSLKDDPSQSANLLAEAKKLNDAQAPK

SEQ ID NO: 44 - protein, 58 aa, Escherichia coli
VDAKFDKEQQMAFYEILHLPNLTEEQRNAFIQSLKDDPSQSANLLAEAKKLNDAQAPK

SEQ ID NO: 45 - protein, 58 aa, Escherichia coli
VDAKFDKEQQVAFYEILHLPNLTEEQRNAFIQSLKDDPSQSANLLAEAKKLNDAQAPK

SEQ ID NO: 46 - protein, 58 aa, Escherichia coli
VDAKFDKEQQAAFYEILHLPNLTEEQRNAFIQSLKDDPSQSANLLAEAKKLNDAQAPK

SEQ ID NO: 47 - protein, 58 aa, Escherichia coli
VDAKFDKEQQHAFYEILHLPNLTEEQRNAFIQSLKDDPSQSANLLAEAKKLNDAQAPK

SEQ ID NO: 48 - protein, 58 aa, Escherichia coli
VDAKFDKEQQRAFYEILHLPNLTEEQRNAFIQSLKDDPSQSANLLAEAKKLNDAQAPK

SEQ ID NO: 49 - protein, 58 aa, Escherichia coli
VDAKFDKEAQEAFYEILHLPNLTEEQRNAFIQSLKDEPSVSKAILAEAKKLNDAQAPK

SEQ ID NO: 50 - protein, 58 aa, Escherichia coli
VDAKFDKEAQEAFYEILHLPNLTEEQRNAFIQSLKDEPSVSRAILAEAKKLNDAQAPK

SEQ ID NO: 51 - protein, 52 aa, Escherichia coli
KEQQNAFYEILHLPNLTEEQRNAFIQSLKDDPSQSANLLAEAKKLNDAQAPK

SEQ ID NO: 52 - protein, 52 aa, Staphylococcus aureus
KEQQNAFYEILHLPNLTEEQRNGFIQSLKDDPSVSKEILAEAKKLNDAQAPK

SEQ ID NO: 53 - protein, 52 aa, Escherichia coli
  misc_feature (3)..(3): Xaa can be any naturally occurring amino acid
  misc_feature (5)..(5): Xaa can be any naturally occurring amino acid
  misc_feature (12)..(12): Xaa can be any naturally occurring amino acid
  misc_feature (22)..(23): Xaa can be any naturally occurring amino acid
  misc_feature (26)..(27): Xaa can be any naturally occurring amino acid
  misc_feature (31)..(31): Xaa can be any naturally occurring amino acid
  misc_feature (34)..(34): Xaa can be any naturally occurring amino acid
  misc_feature (36)..(38): Xaa can be any naturally occurring amino acid
  misc_feature (44)..(45): Xaa can be any naturally occurring amino acid
KEXQXAFYEILXLPNLTEEQRXXFIXXLKDXPSXSXXXLAEAKXXNDAQAPK